European Patent Specification EP 4 012 035 B1, published November 6, 2024. Title: ADENO-ASSOCIATED VIRAL VECTORS FOR TREATING MYOCILIN (MYOC) GLAUCOMA. Applicant: PECHAN, Peter SCARIA, Abraham ARDINGER, Jeffery. Application Not Yet Assigned. The sequence listing filed with the application follows.

SEQUENCE LISTING (24 sequences)

SEQ ID NO: 1 - protein, 272 aa, Homo sapiens
MHLRLISWLFIILNFMEYIGSQNASRGRRQRRMHPNVSQGCQGGCATCSDYNGCLSCKPRLFFALERIGMKQIGVCLSSCPSGYYGTRYPDINKCTKCKADCDTCFNKNFCTKCKSGFYLHLGKCLDNCPEGLEANNHTMECVSIVHCEVSEWNPWSPCTKKGKTCGFKRGTETRVREIIQHPSAKGNLCPPTNETRKCTVQRKKCQKGERGKKGRERKRKKPNKGESKEAIPDSKSLESSKEIPEQRENKQQQKKRKVQDKQKSVSVSTVH

SEQ ID NO: 2 - DNA, 819 bp, Homo sapiens
atgcacttgcgactgatttcttggctttttatcattttgaactttatggaatacatcggcagccaaaacgcctcccggggaaggcgccagcgaagaatgcatcctaacgttagtcaaggctgccaaggaggctgtgcaacatgctcagattacaatggatgtttgtcatgtaagcccagactattttttgctctggaaagaattggcatgaagcagattggagtatgtctctcttcatgtccaagtggatattatggaactcgatatccagatataaataagtgtacaaaatgcaaagctgactgtgatacctgtttcaacaaaaatttctgcacaaaatgtaaaagtggattttacttacaccttggaaagtgccttgacaattgcccagaagggttggaagccaacaaccatactatggagtgtgtcagtattgtgcactgtgaggtcagtgaatggaatccttggagtccatgcacgaagaagggaaaaacatgtggcttcaaaagagggactgaaacacgggtccgagaaataatacagcatccttcagcaaagggtaacctgtgtcccccaacaaatgagacaagaaagtgtacagtgcaaaggaagaagtgtcagaagggagaacgaggaaaaaaaggaagggagaggaaaagaaaaaaacctaataaaggagaaagtaaagaagcaatacctgacagcaaaagtctggaatccagcaaagaaatcccagagcaacgagaaaacaaacagcagcagaagaagcgaaaagtccaagataaacagaaatcggtatcagtcagcactgtacactag

SEQ ID NO: 3 - protein, 502 aa, Homo sapiens
MRFFCARCCSFGPEMPAVQLLLLACLVWDVGARTAQLRKANDQSGRCQYTFSVDNESSCPEQSQAMSVIHNLQRDSSTQRLDLEATKARLSSLESLLHQLTLDQAARPQETQEGLQRELGTLRRERDQLETQTRELETAYSNLLRDKSVLEEEKKRLRQENENLARRLESSSQEVARLRRGQCPQTRDTARAVPPGSREVSTWNLDTLAFQELKSELTEVPASRILKESPSGYLRSGEGDTGCGELVWVGEPLTLRTAETITGKYGVWMRDPKPTYPYTQETTWRIDTVGTDVRQVFEYDLISQFMQGYPSKVHILPRPLESTGAVVYSGSLYFQGAESRTVIRYELNTETVKAEKEIPGAGYHGQFPYSWGGYTDIDLAVDEAGLWVIYSTDEAKGAIVLSKLNPENLELEQTWETNIRKQSVANAFIICGTLYTVSSYTSADATVNFAYDTGTGISKTLTIPFKNRYKYSSMIDYNPLEKKLFAWDNLNMVTYDIKLSKM

SEQ ID NO: 4 - DNA, 1515 bp, Artificial Sequence
  Synthetic Construct
atgaggttcttctgtgcacgttgctgcagctttgggcctgagatgccagctgtccagctgctgcttctggcctgcctggtgtgggatgtgggggccaggacagctcagctcaggaaggccaatgaccagagtggccgatgccagtataccttcagtgtggccagtcccaatgaatccagctgcccagagcagagccaggccatgtcagtcatccataacttacagagagacagcagcacccaacgcttagacctggaggccaccaaagctcgactcagctccctggagagcctcctccaccaattgaccttggaccaggctgccaggccccaggagacccaggaggggctgcagagggagctgggcaccctgaggcgggagcgggaccagctggaaacccaaaccagagagttggagactgcctacagcaacctcctccgagacaagtcagttctggaggaagagaagaagcgactaaggcaagaaaatgagaatctggccaggaggttggaaagcagcagccaggaggtagcaaggctgagaaggggccagtgtccccagacccgagacactgctcgggctgtgccaccaggctccagagaagtttctacgtggaatttggacactttggccttccaggaactgaagtccgagctaactgaagttcctgcttcccgaattttgaaggagagcccatctggctatctcaggagtggagagggagacaccggatgtggagaactagtttgggtaggagagcctctcacgctgagaacagcagaaacaattactggcaagtatggtgtgtggatgcgagaccccaagcccacctacccctacacccaggagaccacgtggagaatcgacacagttggcacggatgtccgccaggtttttgagtatgacctcatcagccagtttatgcagggctacccttctaaggttcacatactgcctaggccactggaaagcacgggtgctgtggtgtactcggggagcctctatttccagggcgctgagtccagaactgtcataagatatgagctgaataccgagacagtgaaggctgagaaggaaatccctggagctggctaccacggacagttcccgtattcttggggtggctacacggacattgacttggctgtggatgaagcaggcctctgggtcatttacagcaccgatgaggccaaaggtgccattgtcctctccaaactgaacccagagaatctggaactcgaacaaacctgggagacaaacatccgtaagcagtcagtcgccaatgccttcatcatctgtggcaccttgtacaccgtcagcagctacacctcagcagatgctaccgtcaactttgcttatgacacaggcacaggtatcagcaagaccctgaccatcccattcaagaaccgctataagtacagcagcatgattgactacaaccccctggagaagaagctctttgcctgggacaacttgaacatggtcacttatgacatcaagctctccaagatgtag

SEQ ID NO: 5 - DNA, 19 bp, Artificial Sequence
  Synthetic Construct
ggccatgtcagtcatccat

SEQ ID NO: 6 - protein, 7 aa, Artificial Sequence
  Synthetic Construct
QAMSVIH

SEQ ID NO: 7 - DNA, 23 bp, Artificial Sequence
  Synthetic Construct
aatagtgaagccacagatgtatt

SEQ ID NO: 8 - protein, 259 aa, Homo sapiens
MRLGLCVVVLSWTHLTISSRGIKGKRQRRISAEGSQACAKGCELCSEVNGCLKCSPKLFILLERNDIRQVGVCLPSCPPGYFDARNPDMNKCIKCKIEHCEACFSHNFCTKCKEGLHKGRCYPACPEGSSAANGTMECSSPAQCEMSEWSPWGPCSKKQQLCGFRRGSEERTRRVLHAPVGDHAACSDTKETRRCTVRRVPCPEGQKRRKGGQGRRENANRNLARKESKEAGAGSRRRKGQQQQQQQGTVGPLTSAGPA

SEQ ID NO: 9 - protein, 243 aa, Homo sapiens
MQFRLFSFALIILNCMDYSHCQGNRWRRSKRASYVSNPICKGCLSCSKDNGCSRCQQKLFFFLRREGMRQYGECLHSCPSGYYGHRAPDMNRCARCRIENCDSCFSKDFCTKCKVGFYLHRGRCFDECPDGFAPLEETMECVEGCEVGHWSEWGTCSRNNRTCGFKWGLETRTRQIVKKPVKDTILCPTIAESRRCKMTMRHCPGGKRTPKAKEKRNKKKKRKLIERAQEQHSVFLATDRANQ

SEQ ID NO: 10 - protein, 234 aa, Homo sapiens
MRAPLCLLLLVAHAVDMLALNRRKKQVGTGLGGNCTGCIICSEENGCSTCQQRLFLFIRREGIRQYGKCLHDCPPGYFGIRGQEVNRCKKCGATCESCFSQDFCIRCKRQFYLYKGKCLPTCPPGTLAHQNTRECQGECELGPWGGWSPCTHNGKTCGSAWGLESRVREAGRAGHEEAATCQVLSESRKCPIQRPCPGERSPGQKKGRKDRRPRKDRKLDRRLDVRPRQPGLQP

SEQ ID NO: 11 - protein, 131 aa, Artificial Sequence
  Synthetic Construct
MRLGLCVVVLSWTHLTISSRGIKGKRQRRISAEGSQACAKGCELCSEVNGCLKCSPKLFILLERNDIRQVGVCLPSCPPGYFDARNPDMNKCIKCKIEHCEACFSHNFCTKCKEGLHKGRCYPACPEGSSA

SEQ ID NO: 12 - protein, 202 aa, Artificial Sequence
  Synthetic Construct
MRLGLCVVVLSWTHLTISSRGIKGKRQRRISAEGSQACAKGCELCSEVNGCLKCSPKLFILLERNDIRQVGVCLPSCPPGYFDARNPDMNKCIKCKIEHCEACFSHNFCTKCKEGLHKGRCYPACPEGSSAANGTMECSSPAQCEMSEWSPWGPCSKKQQLCGFRRGSEERTRRVLHAPVGDHAACSDTKETRRCTVRRVPC

SEQ ID NO: 13 - protein, 134 aa, Artificial Sequence
  Synthetic Construct
MQFRLFSFALIILNCMDYSHCQGNRWRRSKRASYVSNPICKGCLSCSKDNGCSRCQQKLFFFLRREGMRQYGECLHSCPSGYYGHRAPDMNRCARCRIENCDSCFSKDFCTKCKVGFYLHRGRCFDECPDGFAP

SEQ ID NO: 14 - protein, 203 aa, Artificial Sequence
  Synthetic Construct
MQFRLFSFALIILNCMDYSHCQGNRWRRSKRASYVSNPICKGCLSCSKDNGCSRCQQKLFFFLRREGMRQYGECLHSCPSGYYGHRAPDMNRCARCRIENCDSCFSKDFCTKCKVGFYLHRGRCFDECPDGFAPLEETMECVEGCEVGHWSEWGTCSRNNRTCGFKWGLETRTRQIVKKPVKDTILCPTIAESRRCKMTMRHC

SEQ ID NO: 15 - protein, 135 aa, Artificial Sequence
  Synthetic Construct
MHLRLISWLFIILNFMEYIGSQNASRGRRQRRMHPNVSQGCQGGCATCSDYNGCLSCKPRLFFALERIGMKQIGVCLSSCPSGYYGTRYPDINKCTKCKADCDTCFNKNFCTKCKSGFYLHLGKCLDNCPEGLEA

SEQ ID NO: 16 - protein, 146 aa, Artificial Sequence
  Synthetic Construct
MHLRLISWLFIILNFMEYIGSQNASRGRRQRRMHPNVSQGCQGGCATCSDYNGCLSCKPRLFFALERIGMKQIGVCLSSCPSGYYGTRYPDINKCTKCKADCDTCFNKNFCTKCKSGFYLHLGKCLDNCPEGLEANNHTMECVSIV

SEQ ID NO: 17 - protein, 206 aa, Artificial Sequence
  Synthetic Construct
MHLRLISWLFIILNFMEYIGSQNASRGRRQRRMHPNVSQGCQGGCATCSDYNGCLSCKPRLFFALERIGMKQIGVCLSSCPSGYYGTRYPDINKCTKCKADCDTCFNKNFCTKCKSGFYLHLGKCLDNCPEGLEANNHTMECVSIVHCEVSEWNPWSPCTKKGKTCGFKRGTETRVREIIQHPSAKGNLCPPTNETRKCTVQRKKC

SEQ ID NO: 18 - protein, 128 aa, Artificial Sequence
  Synthetic Construct
MRAPLCLLLLVAHAVDMLALNRRKKQVGTGLGGNCTGCIICSEENGCSTCQQRLFLFIRREGIRQYGKCLHDCPPGYFGIRGQEVNRCKKCGATCESCFSQDFCIRCKRQFYLYKGKCLPTCPPGTLA

SEQ ID NO: 19 - protein, 195 aa, Artificial Sequence
  Synthetic Construct
MRAPLCLLLLVAHAVDMLALNRRKKQVGTGLGGNCTGCIICSEENGCSTCQQRLFLFIRREGIRQYGKCLHDCPPGYFGIRGQEVNRCKKCGATCESCFSQDFCIRCKRQFYLYKGKCLPTCPPGTLAHQNTRECQGECELGPWGGWSPCTHNGKTCGSAWGLESRVREAGRAGHEEAATCQVLSESRKCPIQRP

SEQ ID NO: 20 - DNA, 78 bp, Artificial Sequence
  Synthetic Construct
cactccctctctgcgcgctcgctcgctcactgaggccgggcgaccaaaggtcgcccacgcccgggctttgcccgggcg

SEQ ID NO: 21 - DNA, 31 bp, Artificial Sequence
  Synthetic Construct
accacggacagttcctgtattcttggggtgg

SEQ ID NO: 22 - DNA, 31 bp, Artificial Sequence
  Synthetic Construct
ccaccccaagaatacaggaactgtccgtggt

SEQ ID NO: 23 - DNA, 29 bp, Artificial Sequence
  Synthetic Construct
tctgtggcaccttgcacaccgtcagcagc

SEQ ID NO: 24 - DNA, 29 bp, Artificial Sequence
  Synthetic Construct
gctgctgacggtgtgcaaggtgccacaga